European Patent Specification EP 3 160 448 B1, published August 6, 2025. Title: LIPOSOMAL FORMULATIONS FOR DELIVERY OF NUCLEIC ACIDS. Applicant: RAMOT at Tel Aviv University Ltd. The sequence listing filed with the application follows.

SEQUENCE LISTING (8 sequences)

SEQ ID NO: 1 - RNA, 21 nt, Artificial sequence
  siRNA
  modified_base (1)..(1): 2'-O-methylation
  modified_base (2)..(2): 2'-O-methylation
  modified_base (11)..(11): 2'-O-methylation
  modified_base (12)..(12): 2'-O-methylation
  modified_base (14)..(14): 2'-O-methylation
  modified_base (20)..(20): 2'-O-methylation
ugaagaagaucacccuccuua

SEQ ID NO: 2 - DNA, 20 bp, Artificial sequence
  Primer
accagcacgtcgtaggattc

SEQ ID NO: 3 - DNA, 19 bp, Artificial sequence
  Primer
caagcacaattgccgtagg

SEQ ID NO: 4 - DNA, 20 bp, Artificial sequence
  Primer
tcagggtttcacatttggca

SEQ ID NO: 5 - DNA, 21 bp, Artificial sequence
  siRNA
guaggacucucauucgggatt

SEQ ID NO: 6 - DNA, 21 bp, Artificial sequence
  siRNA
  modified_base (1)..(3): 2'-O-Me
  modified_base (5)..(5): 2'-O-Me
  modified_base (7)..(8): 2'-O-Me
  modified_base (12)..(12): 2'-O-Me
  modified_base (14)..(17): 2'-O-Me
  modified_base (20)..(21): phosphorothioate linkage
  modified_base (20)..(21): Deoxyribonucleotide
cuuacgcugaguacuucgatt

SEQ ID NO: 7 - DNA, 21 bp, Artificial sequence
  siRNA
  modified_base (7)..(7): 2'-OMe
  modified_base (11)..(11): 2'-OMe
  modified_base (16)..(16): 2'-OMe
  modified_base (20)..(21): phosphorothioate linkage
  modified_base (20)..(21): Deoxyribonucleotide
ucgaaguacucagcguaagtt

SEQ ID NO: 8 - DNA, 20 bp, Artificial sequence
  Primer
gagcatggatcggaaaacca